European Patent Application EP 4 431 607 A2, published September 18, 2024. Title: HIGH-THROUGHPUT PRECISION GENOME EDITING. Applicant: The Board of Trustees of the Leland Stanford Junior University. Application US. The sequence listing filed with the application follows.

SEQUENCE LISTING (43 sequences)

SEQ ID NO: 1 - DNA, 21 bp, synthetic construct
  misc_feature 1..21: note = Synthetic ADE1 forward primer
  source 1..21: mol_type = other DNA
cattggtggccagaggtaaag

SEQ ID NO: 2 - DNA, 21 bp, synthetic construct
  misc_feature 1..21: note = Synthetic ADE1 reverse primer
  source 1..21: mol_type = other DNA
gtgaggagttacactggcgac

SEQ ID NO: 3 - DNA, 20 bp, synthetic construct
  misc_feature 1..20: note = Synthetic ADE1 guide sequence (20 bp)
  source 1..20: mol_type = other DNA
caagtgcaaagattatgcta

SEQ ID NO: 4 - DNA, 921 bp, synthetic construct
  misc_feature 1..921: note = Synthetic ADE1 sequence
  source 1..921: mol_type = other DNA
atgtcaattacgaagactgaactggacggtatattgccattggtggccagaggtaaagttagagacatatatgaggtagacgctggtacgttgctgtttgttgctacggatcgtatctctgcatatgacgttattatggaaaacagcattcctgaaaaggggatcctattgaccaaactgtcagagttctggttcaagttcctgtccaacgatgttcgtaatcatttggtcgacatcgccccaggtaagactattttcgattatctacctgcaaaattgagcgaaccaaagtacaaaacgcaactagaagaccgctctctattggttcacaaacataaactaattccattggaagtaattgtcagaggctacatcaccggatctgcttggaaagagtacgtaaaaacaggtactgtgcatggtttgaaacaacctcaaggacttaaagaatctcaagagttcccagaaccaatcttcaccccatcgaccaaggctgaacaaggtgaacatgacgaaaacatctctcctgcccaggccgctgagctggtgggtgaagatttgtcacgtagagtggcagaactggctgtaaaactgtactccaagtgcaaagattatgctaaggagaagggcatcatcatcgcagacactaaattcgaattcggtattgacgaaaagaccaatgaaattattctagtggacgaggtgctaacgccagactcctctagattctggaacggtgcctcttataaggtaggagaatcccaagattcttacgataagcaatttttaagagactggcttactgctaataagttgaacggtgttaacggcgtcaaaatgccccaagacattgtcgacaggacaagggccaaatatatagaggcttatgaaacattgacagggtctaaatggtctcactaa

SEQ ID NO: 5 - DNA, 720 bp, synthetic construct
  misc_feature 1..720: note = Synthetic eGFP sequence
  source 1..720: mol_type = other DNA
atggtgagcaagggcgaggagctgttcaccggggtggtgcccatcctggtcgagctggacggcgacgtaaacggccacaagttcagcgtgtccggcgagggcgagggcgatgccacctacggcaagctgaccctgaagttcatctgcaccaccggcaagctgcccgtgccctggcccaccctcgtgaccaccctgacctacggcgtgcagtgcttcagccgctaccccgaccacatgaagcagcacgacttcttcaagtccgccatgcccgaaggctacgtccaggagcgcaccatcttcttcaaggacgacggcaactacaagacccgcgccgaggtgaagttcgagggcgacaccctggtgaaccgcatcgagctgaagggcatcgacttcaaggaggacggcaacatcctggggcacaagctggagtacaactacaacagccacaacgtctatatcatggccgacaagcagaagaacggcatcaaggtgaacttcaagatccgccacaacatcgaggacggcagcgtgcagctcgccgaccactaccagcagaacacccccatcggcgacggccccgtgctgctgcccgacaaccactacctgagcacccagtccgccctgagcaaagaccccaacgagaagcgcgatcacatggtcctgctggagttcgtgaccgccgccgggatcactctcggcatggacgagctgtacaagtaa

SEQ ID NO: 6 - DNA, 45 bp, synthetic construct
  misc_feature 1..45: note = Synthetic Fusion linker sequence
  source 1..45: mol_type = other DNA
ggtggaggaggctctggtggaggcggtagcggaggcggagggtcg

SEQ ID NO: 7 - DNA, 50 bp, synthetic construct
  misc_feature 1..50: note = Synthetic ADE1 homology arm
  source 1..50: mol_type = other DNA
tagagtggcagaactggctgtaaaactgtactccaagtgcaaagattatg

SEQ ID NO: 8 - DNA, 38 bp, synthetic construct
  misc_feature 1..38: note = Synthetic Donor sequence
  source 1..38: mol_type = other DNA
gttcacactcactagagtgacgaacaatacacgttagc

SEQ ID NO: 9 - DNA, 50 bp, synthetic construct
  misc_feature 1..50: note = Synthetic ADE1 homology arm
  source 1..50: mol_type = other DNA
ctaaggagaagggcatcatcatcgcagacactaaattcgaattcggtatt

SEQ ID NO: 10 - DNA, 1716 bp, synthetic construct
  misc_feature 1..1716: note = Synthetic ADE2 sequence
  source 1..1716: mol_type = other DNA
atggattctagaacagttggtatattaggagggggacaattgggacgtatgattgttgaggcagcaaacaggctcaacattaagacggtaatactagatgctgaaaattctcctgccaaacaaataagcaactccaatgaccacgttaatggctccttttccaatcctcttgatatcgaaaaactagctgaaaaatgtgatgtgctaacgattgagattgagcatgttgatgttcctacactaaagaatcttcaagtaaaacatcccaaattaaaaatttacccttctccagaaacaatcagattgatacaagacaaatatattcaaaaagagcatttaatcaaaaatggtatagcagttacccaaagtgttcctgtggaacaagccagtgagacgtccctattgaatgttggaagagatttgggttttccattcgtcttgaagtcgaggactttggcatacgatggaagaggtaacttcgttgtaaagaataaggaaatgattccggaagctttggaagtactgaaggatcgtcctttgtacgccgaaaaatgggcaccatttactaaagaattagcagtcatgattgtgagatctgttaacggtttagtgttttcttacccaattgtagagactatccacaaggacaatatttgtgacttatgttatgcgcctgctagagttccggactccgttcaacttaaggcgaagttgttggcagaaaatgcaatcaaatcttttcccggttgtggtatatttggtgtggaaatgttctatttagaaacaggggaattgcttattaacgaaattgccccaaggcctcacaactctggacattataccattgatgcttgcgtcacttctcaatttgaagctcatttgagatcaatattggatttgccaatgccaaagaatttcacatctttctccaccattacaacgaacgccattatgctaaatgttcttggagacaaacatacaaaagataaagagctagaaacttgcgaaagagcattggcgactccaggttcctcagtgtacttatatggaaaagagtctagacctaacagaaaagtaggtcacataaatattattgcctccagtatggcggaatgtgaacaaaggctgaactacattacaggtagaactgatattccaatcaaaatctctgtcgctcaaaagttggacttggaagcaatggtcaaaccattggttggaatcatcatgggatcagactctgacttgccggtaatgtctgccgcatgtgcggttttaaaagattttggcgttccatttgaagtgacaatagtctctgctcatagaactccacataggatgtcagcatatgctatttccgcaagcaagcgtggaattaaaacaattatcgctggagctggtggggctgctcacttgccaggtatggtggctgcaatgacaccacttcctgtcatcggtgtgcccgtaaaaggttcttgtctagatggagtagattctttacattcaattgtgcaaatgcctagaggtgttccagtagctaccgtcgctattaataatagtacgaacgctgcgctgttggctgtcagactgcttggcgcttatgattcaagttatacaacgaaaatggaacagtttttattaaagcaagaagaagaagttcttgtcaaagcacaaaagttagaaactgtcggttacgaagcttatctagaaaacaagtaa

SEQ ID NO: 11 - DNA, 50 bp, synthetic construct
  misc_feature 1..50: note = Synthetic ADE2 homology arm
  source 1..50: mol_type = other DNA
tggaaatgttctatttagaaacaggggaattgcttattaacgaaattgcc

SEQ ID NO: 12 - DNA, 50 bp, synthetic construct
  misc_feature 1..50: note = Synthetic ADE2 homology arm
  source 1..50: mol_type = other DNA
tgaaggcctcacaactctggacattataccattgatgcttgcgtcacttc

SEQ ID NO: 13 - DNA, 18 bp, synthetic construct
  misc_feature 1..18: note = Synthetic Guide 3 0.74
  source 1..18: mol_type = other DNA
attaacgaaattgcccca

SEQ ID NO: 14 - DNA, 1338 bp, synthetic construct
  misc_feature 1..1338: note = Synthetic Retron Ec86 sequence
  source 1..1338: mol_type = other DNA
taactatgataagattccgtatgcgcacccttagcgagaggtttatcattaaggtcaacctctggatgttgtttcggcatcctgcattgaatctgagttactgtctgttttccttgttggaacggagagcatcgcctgatgctctccgagccaaccaggaaacccgttttttctgacgtaagggtgcgcaactttcatgaaatccgctgaatatttgaacacttttagattgagaaatctcggcctacctgtcatgaacaatttgcatgacatgtctaaggcgactcgcatatctgttgaaacacttcggttgttaatctatacagctgattttcgctataggatctacactgtagaaaagaaaggcccagagaagagaatgagaaccatttaccaaccttctcgagaacttaaagccttacaaggatgggttctacgtaacattttagataaactgtcgtcatctcctttttctattggatttgaaaagcaccaatctattttgaataatgctaccccgcatattggggcaaactttatactgaatattgatttggaggattttttcccaagtttaactgctaacaaagtttttggagtgttccattctcttggttataatcgactaatatcttcagttttgacaaaaatatgttgttataaaaatctgctaccacaaggtgctccatcatcacctaaattagctaatctaatatgttctaaacttgattatcgtattcagggttatgcaggtagtcggggcttgatatatacgagatatgccgatgatctcaccttatctgcacagtctatgaaaaaggttgttaaagcacgtgattttttattttctataatcccaagtgaaggattggttattaactcaaaaaaaacttgtattagtgggcctcgtagtcagaggaaagttacaggtttagttatttcacaagagaaagttgggataggtagagaaaaatataaagaaattagagcaaagatacatcatatattttgcggtaagtcttctgagatagaacacgttaggggatggttgtcatttattttaagtgtggattcaaaaagccataggagattaataacttatattagcaaattagaaaaaaaatatggaaagaaccctttaaataaagcgaagacctaatggtcttcgttttaaaactaaagctcataggttgaaaaattgagcacttcttcgtccaaccagttatttagttcctgcaatcgtttctgcaggggcatcaattcgtttcttacgaataccttgctagccttctccacatccccaaaccccccgacattattaggcataattcccatcat

SEQ ID NO: 15 - DNA, 20 bp, synthetic construct
  misc_feature 1..20: note = Synthetic Plasmid start sequence
  source 1..20: mol_type = other DNA
taactatgataagattccgt

SEQ ID NO: 16 - DNA, 12 bp, synthetic construct
  misc_feature 1..12: note = Synthetic Inverted repeat sequence
  source 1..12: mol_type = other DNA
tgcgcaccctta

SEQ ID NO: 17 - DNA, 12 bp, synthetic construct
  misc_feature 1..12: note = Synthetic Second inverted repeat
  source 1..12: mol_type = other DNA
taagggtgcgca

SEQ ID NO: 18 - DNA, 82 bp, synthetic construct
  misc_feature 1..82: note = Synthetic msr locus
  source 1..82: mol_type = other DNA
atgcgcacccttagcgagaggtttatcattaaggtcaacctctggatgttgtttcggcatcctgcattgaatctgagttact

SEQ ID NO: 19 - DNA, 86 bp, synthetic construct
  misc_feature 1..86: note = Synthetic msd locus
  source 1..86: mol_type = other DNA
tctgagttactgtctgttttccttgttggaacggagagcatcgcctgatgctctccgagccaaccaggaaacccgttttttctgac

SEQ ID NO: 20 - DNA, 41 bp, synthetic construct
  misc_feature 1..41: note = Synthetic Replaceable region
  source 1..41: mol_type = other DNA
tgttggaacggagagcatcgcctgatgctctccgagccaac

SEQ ID NO: 21 - DNA, 963 bp, synthetic construct
  misc_feature 1..963: note = Synthetic Ec86 reverse transcriptase (optimized)
  source 1..963: mol_type = other DNA
atgaaatccgctgaatatttgaacacttttagattgagaaatctcggcctacctgtcatgaacaatttgcatgacatgtctaaggcgactcgcatatctgttgaaacacttcggttgttaatctatacagctgattttcgctataggatctacactgtagaaaagaaaggcccagagaagagaatgagaaccatttaccaaccttctcgagaacttaaagccttacaaggatgggttctacgtaacattttagataaactgtcgtcatctcctttttctattggatttgaaaagcaccaatctattttgaataatgctaccccgcatattggggcaaactttatactgaatattgatttggaggattttttcccaagtttaactgctaacaaagtttttggagtgttccattctcttggttataatcgactaatatcttcagttttgacaaaaatatgttgttataaaaatctgctaccacaaggtgctccatcatcacctaaattagctaatctaatatgttctaaacttgattatcgtattcagggttatgcaggtagtcggggcttgatatatacgagatatgccgatgatctcaccttatctgcacagtctatgaaaaaggttgttaaagcacgtgattttttattttctataatcccaagtgaaggattggttattaactcaaaaaaaacttgtattagtgggcctcgtagtcagaggaaagttacaggtttagttatttcacaagagaaagttgggataggtagagaaaaatataaagaaattagagcaaagatacatcatatattttgcggtaagtcttctgagatagaacacgttaggggatggttgtcatttattttaagtgtggattcaaaaagccataggagattaataacttatattagcaaattagaaaaaaaatatggaaagaaccctttaaataaagcgaagacctaa

SEQ ID NO: 22 - skipped

SEQ ID NO: 23 - DNA, 179 bp, synthetic construct
  misc_feature 1..179: note = Synthetic Sequence located 3' of EC86 reverse transcriptase sequence
  source 1..179: mol_type = other DNA
tggtcttcgttttaaaactaaagctcataggttgaaaaattgagcacttcttcgtccaaccagttatttagttcctgcaatcgtttctgcaggggcatcaattcgtttcttacgaataccttgctagccttctccacatccccaaaccccccgacattattaggcataattcccatcat

SEQ ID NO: 24 - DNA, 669 bp, synthetic construct
  misc_feature 1..669: note = Synthetic Cassette sequence
  source 1..669: mol_type = other DNA
gttcctggccttttgctggccttttgctcttaattaagtatatgtgttatgtagtatactctttcttcaacaattaaatactctcggtagccaagttggtttaaggcgcaagactgtaatttatcactacgaaatcttgagatcgggcgttcgactcgcccccgggagagatggccggcatggtcccagcctcctcgctggcgccggctgggcaacaccttcgggtggcgaatgggactttatgcgcacccttagcgagaggtttatcattaaggtcaacctctggatgttgtttcggcatcctgcattgaatctgagttactgtctgttttcctctctgacaattacttccaatggaattagtttatgtttgtgaaccaatagagatcagtcttctagttgcgttttgtactttggttcgctcaattttgcaggaggaaacccgtttcttctgacgtaagggtgcgcagtttgtgaaccaatagagaggttttagagctagaaatagcaagttaaaataaggctagtccgttatcaacttgaaaaagtggcaccgagtcggtgctttttttattttttgtcactattgttatgtaaaatgccacctctgacagtatggaacgcaaacttctgtctagtggataggaactcttgttgttctttgctagc

SEQ ID NO: 25 - skipped

SEQ ID NO: 26 - DNA, 20 bp, synthetic construct
  misc_feature 1..20: note = Synthetic Pci1-Up sequence (primer binding site)
  source 1..20: mol_type = other DNA
cttttgctggccttttgctc

SEQ ID NO: 27 - skipped

SEQ ID NO: 28 - DNA, 132 bp, synthetic construct
  misc_feature 1..132: note = Synthetic tRNA-Tyr
  source 1..132: mol_type = other DNA
gtatatgtgttatgtagtatactctttcttcaacaattaaatactctcggtagccaagttggtttaaggcgcaagactgtaatttatcactacgaaatcttgagatcgggcgttcgactcgcccccgggaga

SEQ ID NO: 29 - DNA, 72 bp, synthetic construct
  misc_feature 1..72: note = Synthetic HDV ribozyme
  source 1..72: mol_type = other DNA
gatggccggcatggtcccagcctcctcgctggcgccggctgggcaacaccttcgggtggcgaatgggacttt

SEQ ID NO: 30 - DNA, 121 bp, synthetic construct
  misc_feature 1..121: note = Synthetic msd locus
  source 1..121: mol_type = other DNA
ctctgacaattacttccaatggaattagtttatgtttgtgaaccaatagagatcagtcttctagttgcgttttgtactttggttcgctcaattttgcaggaggaaacccgttttttctgac

SEQ ID NO: 31 - DNA, 23 bp, synthetic construct
  misc_feature 1..23: note = Synthetic msd locus (portion overlaping the vector, not including donor)
  source 1..23: mol_type = other DNA
tctgagttactgtctgttttcct

SEQ ID NO: 32 - DNA, 94 bp, synthetic construct
  misc_feature 1..94: note = Synthetic Vector sequence
  source 1..94: mol_type = other DNA
atgcgcacccttagcgagaggtttatcattaaggtcaacctctggatgttgtttcggcatcctgcattgaatctgagttactgtctgttttcct

SEQ ID NO: 33 - DNA, 100 bp, synthetic construct
  misc_feature 1..100: note = Synthetic Donor DNA1
  source 1..100: mol_type = other DNA
ctctgacaattacttccaatggaattagtttatgtttgtgaaccaatagagatcagtcttctagttgcgttttgtactttggttcgctcaattttgcagg

SEQ ID NO: 34 - DNA, 34 bp, synthetic construct
  misc_feature 1..34: note = Synthetic Constant synthesis sequence
  source 1..34: mol_type = other DNA
aggaaacccgttttttctgacgtaagggtgcgca

SEQ ID NO: 35 - DNA, 20 bp, synthetic construct
  misc_feature 1..20: note = Synthetic Guide2 sequence
  source 1..20: mol_type = other DNA
gtttgtgaaccaatagagag

SEQ ID NO: 36 - DNA, 82 bp, synthetic construct
  misc_feature 1..82: note = Synthetic sgRNA coding sequence
  source 1..82: mol_type = other DNA
gttttagagctagaaatagcaagttaaaataaggctagtccgttatcaacttgaaaaagtggcaccgagtcggtgctttttt

SEQ ID NO: 37 - DNA, 75 bp, synthetic construct
  misc_feature 1..75: note = Synthetic SNR52 terminator
  source 1..75: mol_type = other DNA
tttattttttgtcactattgttatgtaaaatgccacctctgacagtatggaacgcaaacttctgtctagtggata

SEQ ID NO: 38 - DNA, 19 bp, synthetic construct
  misc_feature 1..19: note = Synthetic RPR1 terminator
  source 1..19: mol_type = other DNA
ggaactcttgttgttcttt

SEQ ID NO: 39 - skipped

SEQ ID NO: 40 - protein, 15 aa, synthetic construct
  REGION 1..15: note = Synthetic Partial ADE1 amino acid sequence (N-terminal to edit site)
PAKLSEPKYKTQLED

SEQ ID NO: 41 - protein, 17 aa, synthetic construct
  REGION 1..17: note = Synthetic Partial ADE1 amino acid sequence (C-terminal to edit site)
SLLVHKHKLIPLEVIVR

SEQ ID NO: 42 - DNA, 1338 bp, synthetic construct
  source 1..1338: mol_type = other DNA
attgatactattctaaggcatacgcgtgggaatcgctctccaaatagtaattccagttggagacctacaacaaagccgtaggacgtaacttagactcaatgacagacaaaaggaacaaccttgcctctcgtagcggactacgagaggctcggttggtcctttgggcaaaaaagactgcattcccacgcgttgaaagtactttaggcgacttataaacttgtgaaaatctaactctttagagccggatggacagtacttgttaaacgtactgtacagattccgctgagcgtatagacaactttgtgaagccaacaattagatatgtcgactaaaagcgatatcctagatgtgacatcttttctttccgggtctcttctcttactcttggtaaatggttggaagagctcttgaatttcggaatgttcctacccaagatgcattgtaaaatctatttgacagcagtagaggaaaaagataacctaaacttttcgtggttagataaaacttattacgatggggcgtataaccccgtttgaaatatgacttataactaaacctcctaaaaaagggttcaaattgacgattgtttcaaaaacctcacaaggtaagagaaccaatattagctgattatagaagtcaaaactgtttttatacaacaatatttttagacgatggtgttccacgaggtagtagtggatttaatcgattagattatacaagatttgaactaatagcataagtcccaatacgtccatcagccccgaactatatatgctctatacggctactagagtggaatagacgtgtcagatactttttccaacaatttcgtgcactaaaaaataaaagatattagggttcacttcctaaccaataattgagttttttttgaacataatcacccggagcatcagtctcctttcaatgtccaaatcaataaagtgttctctttcaaccctatccatctctttttatatttctttaatctcgtttctatgtagtatataaaacgccattcagaagactctatcttgtgcaatcccctaccaacagtaaataaaattcacacctaagtttttcggtatcctctaattattgaatataatcgtttaatcttttttttatacctttcttgggaaatttatttcgcttctggattaccagaagcaaaattttgatttcgagtatccaactttttaactcgtgaagaagcaggttggtcaataaatcaaggacgttagcaaagacgtccccgtagttaagcaaagaatgcttatggaacgatcggaagaggtgtaggggtttggggggctgtaataatccgtattaagggtagta

SEQ ID NO: 43 - DNA, 669 bp, synthetic construct
  source 1..669: mol_type = other DNA
caaggaccggaaaacgaccggaaaacgagaattaattcatatacacaatacatcatatgagaaagaagttgttaatttatgagagccatcggttcaaccaaattccgcgttctgacattaaatagtgatgctttagaactctagcccgcaagctgagcgggggccctctctaccggccgtaccagggtcggaggagcgaccgcggccgacccgttgtggaagcccaccgcttaccctgaaatacgcgtgggaatcgctctccaaatagtaattccagttggagacctacaacaaagccgtaggacgtaacttagactcaatgacagacaaaaggagagactgttaatgaaggttaccttaatcaaatacaaacacttggttatctctagtcagaagatcaacgcaaaacatgaaaccaagcgagttaaaacgtcctcctttgggcaaagaagactgcattcccacgcgtcaaacacttggttatctctccaaaatctcgatctttatcgttcaattttattccgatcaggcaatagttgaactttttcaccgtggctcagccacgaaaaaaataaaaaacagtgataacaatacattttacggtggagactgtcataccttgcgtttgaagacagatcacctatccttgagaacaacaagaaacgatcg